European Patent Application EP 4 692 353 A1, published February 11, 2026. Title: Recombinant protein. Applicant: Kikkoman Corporation. The sequence listing filed with the application follows.

SEQUENCE LISTING (45 sequences)

SEQ ID NO: 1 - DNA, 24 bp, synthetic construct
  misc_feature 1..24: note = primer
  source 1..24: mol_type = other DNA
tgagtttatctgactaaatcttag

SEQ ID NO: 2 - DNA, 25 bp, synthetic construct
  misc_feature 1..25: note = primer
  source 1..25: mol_type = other DNA
ggtaccaagctttaaattcgaacag

SEQ ID NO: 3 - protein, 1019 aa, synthetic construct
  REGION 1..1019: note = FCv amino acid sequence
MVLASFLVSGLVLGLLAQQMHPVQSRGVDLGLCDDTRFECKCGDPGYVFNIPVKQCTYFYRWRPYCKPCDKLEAKDVCPKYKRCQECRAGLDSCVGCPPNKYGTWCSGECQCKNGGICDQRTGACACRDRYEGLHCEILRGCPLLNSDTQVQEVKNPPQDPQTIDYSCPPGFKLKGVARINCLPNGQWSSFPPKCIRECSMVSSLEHGKVTSLSAELIEGATLRFSCDSPHYLIGQETLTCQGNGQWSGQIPQCQKLVFCPDLDPVSHAEHKVKIGLEQKYGQFPQGTEVTYTCTGNYFLMGLDTLKCNLDGSWSGTQPSCVKVADREVSCDSKAVDFLDDVGEPVRIHCPAGCSLTAGTVWGTAIYHELSSVCRAAIHAGKVPNSGGAVHVVNNGPYSDFLASDLNGIKSDELKSLAQSFRFDYVRSSTAGKSGCPDGWFEIDENCVYVTSKQRAWERAQGVCTNMAARLAVLDKDVIPSSLTETLRGKGLSTTWIGLHRLDADNHFLWELMDRSTVALNDQLTFWAPGEPGNETNCVYMDIQDQLQSVWKTKSCFQPSSFVCMMDLSDKNKAKCEDPGPLENGHAKLHGQSIDGFYAGSSVRYSCEVLHYLSGTETVSCTSNGTWSAPKPRCIKVITCQTPPVPSYGSVDIKPPSRTNSISRVGSPFLRLPRLPLPLARAAGPPPKPRSAPPSTVDLSSKVKLPEGHYRVGSQAIYTCESRYYELLGSQGRRCDSNGKWSGRPASCIPVCGRSDSPRSPFIVNGNSTEIGQWPWQAGISRWLADHNMWFLLCGGALLNEKWIITAAHCVTYSATAEIIDPSQFKFYLGKYYRDDSKDDDYVQVRTAQEIHVNPNYDPGRLDADIALIQLEESVALTTRVQPICLPTDRSSRNNLKEGHKAVVTGWGLNENETYSEMIQQAVLPVVSASTCEQGYRSSGVPLTVTENMFCAGYKNGRYDSCSGDSGGPLVFSDESRTDRRWVLEGIISWGSVNGCGKANQYAGFTKVNVFLSWIRQFI

SEQ ID NO: 4 - DNA, 3060 bp, synthetic construct
  misc_feature 1..3060: note = FCv nucleotide sequence
  source 1..3060: mol_type = other DNA
atggtgctggctagcttcctggtgtctggactggtgctgggactgctggctcagcaaatgcaccctgtgcagtctcgtggtgtcgacctgggattgtgcgacgacactcgtttcgagtgcaagtgcggcgaccccggttacgtgttcaacatcccagtgaagcagtgcacctacttctaccgttggcgcccctactgcaagccctgcgacaagttggaagctaaggacgtgtgccccaagtacaagcgttgccaagagtgccgtgctggcctggactcctgtgttggttgccctcctaacaaatacggcacctggtgctctggcgagtgccagtgcaagaacggtggtatctgcgaccagcgtaccggtgcttgcgcttgccgtgatcgttacgagggtctgcactgcgagatcctgcgtggttgccctctgctgaactctgacacccaggtgcaagaagtgaagaaccctccacaggaccctcagaccatcgactactcttgccctcccggtttcaagctgaagggtgtcgctcgtatcaactgcctgcctaacggccagtggtctagcttcccacctaagtgcatccgcgagtgctccatggtgtcctcactcgagcacggcaaagtgacctctctgtccgctgagctgatcgagggtgctaccttgaggttctcctgcgactcccctcactacctgatcggtcaagagactctgacctgccaaggcaacggacagtggagcggtcaaatccctcagtgccaaaagctggtgttctgccccgacttggaccccgtgtctcacgctgaacacaaggtgaagatcggcctcgagcagaagtacggacagttccctcagggcaccgaagtgacctacacctgtaccggcaactacttcctgatgggcctcgacaccctgaagtgcaacctggacggttcttggagcggtactcagccctcctgcgtgaaagtggctgaccgtgaagtgtcctgcgactctaaggctgtggacttcctggacgacgtgggagagcctgtgcgtattcactgtcctgctggttgctccctgaccgctggtactgtttggggcaccgctatctaccacgagctgtcctctgtgtgccgcgctgctattcacgctggaaaggtgcccaactccggtggtgctgtgcacgtggtcaacaacggtccctactccgacttcctcgcttccgacctgaacggtatcaagtccgacgagctgaagtccctggctcagtccttccgtttcgactacgtgcgttcctccaccgctggaaagtctggttgtcctgacggatggttcgagatcgacgagaactgcgtgtacgtgacctccaagcagagagcttgggaacgcgctcaaggcgtgtgcaccaatatggctgctcgtctggctgtgctggacaaggacgtgatcccttccagcctgactgagactctgcgtggaaagggactctccaccacctggatcggactgcaccgtttggacgctgacaaccacttcctgtgggagctgatggaccgttccaccgtggctctgaacgaccagctgactttctgggctcctggcgagcctggcaacgagactaactgcgtctacatggacatccaggaccagctgcagtccgtgtggaaaactaagtcctgcttccagccatcctccttcgtgtgcatgatggacctgtccgacaagaacaaggctaagtgcgaggaccccggtcctctcgagaacggtcacgctaagctgcacggccagtccatcgacggtttctacgctggttcctctgtgcgctactcctgcgaggtgctgcactacctgtccggaaccgagactgtgtcctgcacctccaacggaacttggagcgcacctaagcctcgttgcatcaaagtgatcacctgtcagacccctccagtgccttcctacggttccgtggacatcaagccaccttctcgtaccaactccatctctcgtgtgggttctcccttcctgcgtctgcctcgtttgcctctgcctttggctagagctgctggtccacctcctaagccacgttccgctcctccatctaccgtggacttgtcctccaaagtgaagctgcccgagggccactaccgtgtcggttcccaggctatctacacttgcgagtcccgctactacgaactgctgggttctcagggtcgtcgttgcgactcaaatggcaagtggagtggtcgtcccgcttcttgcatccctgtgtgcggtcgttctgactcccctcgttctcctttcatcgtgaacggcaactccaccgagatcggccaatggccttggcaagctggtatctccagatggctggctgaccacaacatgtggttcttgctgtgcggtggcgctctgctgaacgagaagtggatcatcaccgctgctcactgcgtgacctactccgctaccgctgagatcatcgacccctctcagttcaagttctacctgggcaagtactaccgtgacgactccaaggacgacgactacgtccaagtgcgcaccgctcaggagatccacgtgaaccctaactacgaccccggccgtctggacgctgatatcgctctgatccagctcgaggagtctgtcgctctgaccaccagggtgcagcctatctgcttgcctaccgaccgttcctcccgcaacaacctgaaagagggtcacaaggctgtcgtgaccggatggggactcaacgagaacgagacctactctgagatgatccagcaggccgtgctgccagtggtgtccgcttctacttgcgagcagggttaccgttcctccggagtgcctctgactgtgaccgaaaacatgttctgcgctggttacaagaacggccgttacgactcctgctcaggcgattctggtggtcccctggtgttctccgacgagtctcgtactgatcgtcgttgggtgctcgagggtatcatctcctggggttctgtgaacggttgcggcaaggctaaccagtacgctggttttaccaaagtcaacgtgttcctgtcctggatccgtcagttcatctga

SEQ ID NO: 5 - DNA, 25 bp, synthetic construct
  misc_feature 1..25: note = homologous sequence
  source 1..25: mol_type = other DNA
ctgttcgaatttaaagcttggtacc

SEQ ID NO: 6 - DNA, 24 bp, synthetic construct
  misc_feature 1..24: note = homologous sequence
  source 1..24: mol_type = other DNA
tgagtttatctgactaaatcttag

SEQ ID NO: 7 - DNA, 30 bp, synthetic construct
  misc_feature 1..30: note = primer
  source 1..30: mol_type = other DNA
cagtccttccgtctcgactacgtgcgttcc

SEQ ID NO: 8 - DNA, 30 bp, synthetic construct
  misc_feature 1..30: note = primer
  source 1..30: mol_type = other DNA
acggaaggactgagccagggacttcagctc

SEQ ID NO: 9 - DNA, 30 bp, synthetic construct
  misc_feature 1..30: note = primer
  source 1..30: mol_type = other DNA
actaagtcctgcctccagccatcctccttc

SEQ ID NO: 10 - DNA, 30 bp, synthetic construct
  misc_feature 1..30: note = primer
  source 1..30: mol_type = other DNA
gcaggacttagttttccacacggactgcag

SEQ ID NO: 11 - DNA, 30 bp, synthetic construct
  misc_feature 1..30: note = primer
  source 1..30: mol_type = other DNA
gtgggttctccctacctgcgtctgcctcgt

SEQ ID NO: 12 - DNA, 30 bp, synthetic construct
  misc_feature 1..30: note = primer
  source 1..30: mol_type = other DNA
gggagaacccacacgagagatggagttggt

SEQ ID NO: 13 - DNA, 30 bp, synthetic construct
  misc_feature 1..30: note = primer
  source 1..30: mol_type = other DNA
tctggtggtcccgcggtgttctccgacgag

SEQ ID NO: 14 - DNA, 30 bp, synthetic construct
  misc_feature 1..30: note = primer
  source 1..30: mol_type = other DNA
gggaccaccagaatcgcctgagcaggagtc

SEQ ID NO: 15 - DNA, 30 bp, synthetic construct
  misc_feature 1..30: note = primer
  source 1..30: mol_type = other DNA
tctggtggtcccgtggtgttctccgacgag

SEQ ID NO: 16 - DNA, 30 bp, synthetic construct
  misc_feature 1..30: note = primer
  source 1..30: mol_type = other DNA
cccgcggtgttcgtcgacgagtctcgtact

SEQ ID NO: 17 - DNA, 30 bp, synthetic construct
  misc_feature 1..30: note = primer
  source 1..30: mol_type = other DNA
gaacaccgcgggaccaccagaatcgcctga

SEQ ID NO: 18 - DNA, 30 bp, synthetic construct
  misc_feature 1..30: note = primer
  source 1..30: mol_type = other DNA
cccgcggtgttcatcgacgagtctcgtact

SEQ ID NO: 19 - DNA, 30 bp, synthetic construct
  misc_feature 1..30: note = primer
  source 1..30: mol_type = other DNA
cccgcggtgttcttagacgagtctcgtact

SEQ ID NO: 20 - DNA, 30 bp, synthetic construct
  misc_feature 1..30: note = primer
  source 1..30: mol_type = other DNA
ttccgtttcgacttcgtgcgttcctccacc

SEQ ID NO: 21 - DNA, 30 bp, synthetic construct
  misc_feature 1..30: note = primer
  source 1..30: mol_type = other DNA
gtcgaaacggaaggactgagccagggactt

SEQ ID NO: 22 - DNA, 30 bp, synthetic construct
  misc_feature 1..30: note = primer
  source 1..30: mol_type = other DNA
tcctctgtgcgcttctcctgcgaggtgctg

SEQ ID NO: 23 - DNA, 30 bp, synthetic construct
  misc_feature 1..30: note = primer
  source 1..30: mol_type = other DNA
gcgcacagaggaaccagcgtagaaaccgtc

SEQ ID NO: 24 - DNA, 30 bp, synthetic construct
  misc_feature 1..30: note = primer
  source 1..30: mol_type = other DNA
tacctgggcaagttctaccgtgacgactcc

SEQ ID NO: 25 - DNA, 30 bp, synthetic construct
  misc_feature 1..30: note = primer
  source 1..30: mol_type = other DNA
cttgcccaggtagaacttgaactgagaggg

SEQ ID NO: 26 - DNA, 30 bp, synthetic construct
  misc_feature 1..30: note = primer
  source 1..30: mol_type = other DNA
ctgggcaagtacttccgtgacgactccaag

SEQ ID NO: 27 - DNA, 30 bp, synthetic construct
  misc_feature 1..30: note = primer
  source 1..30: mol_type = other DNA
gtacttgcccaggtagaacttgaactgaga

SEQ ID NO: 28 - DNA, 30 bp, synthetic construct
  misc_feature 1..30: note = primer
  source 1..30: mol_type = other DNA
aaggacgacgacaaagtccaagtgcgcacc

SEQ ID NO: 29 - DNA, 30 bp, synthetic construct
  misc_feature 1..30: note = primer
  source 1..30: mol_type = other DNA
gtcgtcgtccttggagtcgtcacggtagta

SEQ ID NO: 30 - DNA, 30 bp, synthetic construct
  misc_feature 1..30: note = primer
  source 1..30: mol_type = other DNA
gaggagtctgtccgtctgaccaccagggtg

SEQ ID NO: 31 - DNA, 30 bp, synthetic construct
  misc_feature 1..30: note = primer
  source 1..30: mol_type = other DNA
gacagactcctcgagctggatcagagcgat

SEQ ID NO: 32 - DNA, 30 bp, synthetic construct
  misc_feature 1..30: note = primer
  source 1..30: mol_type = other DNA
cgcaacaacctgcaagagggtcacaaggct

SEQ ID NO: 33 - DNA, 30 bp, synthetic construct
  misc_feature 1..30: note = primer
  source 1..30: mol_type = other DNA
caggttgttgcgggaggaacggtcggtagg

SEQ ID NO: 34 - DNA, 30 bp, synthetic construct
  misc_feature 1..30: note = primer
  source 1..30: mol_type = other DNA
aacgagaacgagcgctactctgagatgatc

SEQ ID NO: 35 - DNA, 30 bp, synthetic construct
  misc_feature 1..30: note = primer
  source 1..30: mol_type = other DNA
ctcgttctcgttgagtccccatccggtcac

SEQ ID NO: 36 - DNA, 30 bp, synthetic construct
  misc_feature 1..30: note = primer
  source 1..30: mol_type = other DNA
gtggtgtccgctgatacttgcgagcagggt

SEQ ID NO: 37 - DNA, 30 bp, synthetic construct
  misc_feature 1..30: note = primer
  source 1..30: mol_type = other DNA
agcggacaccactggcagcacggcctgctg

SEQ ID NO: 38 - DNA, 30 bp, synthetic construct
  misc_feature 1..30: note = primer
  source 1..30: mol_type = other DNA
gtggtgtccgctgaaacttgcgagcagggt

SEQ ID NO: 39 - DNA, 30 bp, synthetic construct
  misc_feature 1..30: note = primer
  source 1..30: mol_type = other DNA
gtggtgtccgctaaaacttgcgagcagggt

SEQ ID NO: 40 - DNA, 30 bp, synthetic construct
  misc_feature 1..30: note = primer
  source 1..30: mol_type = other DNA
tgcgctggttacgagaacggccgttacgac

SEQ ID NO: 41 - DNA, 30 bp, synthetic construct
  misc_feature 1..30: note = primer
  source 1..30: mol_type = other DNA
gtaaccagcgcagaacatgttttcggtcac

SEQ ID NO: 42 - DNA, 30 bp, synthetic construct
  misc_feature 1..30: note = primer
  source 1..30: mol_type = other DNA
gtcgacgagtctgaaactgatcgtcgttgg

SEQ ID NO: 43 - DNA, 30 bp, synthetic construct
  misc_feature 1..30: note = primer
  source 1..30: mol_type = other DNA
agactcgtcgacgaacaccgcgggaccacc

SEQ ID NO: 44 - DNA, 30 bp, synthetic construct
  misc_feature 1..30: note = primer
  source 1..30: mol_type = other DNA
aacgtgttcctggactggatccgtcagttc

SEQ ID NO: 45 - DNA, 30 bp, synthetic construct
  misc_feature 1..30: note = primer
  source 1..30: mol_type = other DNA
caggaacacgttgactttggtaaaaccagc